European Patent Application EP 4 434 999 A1, published September 25, 2024. Title: SIRPα变体及其应用. Applicant: 杭州尚健生物技术有限公司. The sequence listing filed with the application follows.

SEQUENCE LISTING (27 sequences)

SEQ ID NO: 1 - protein, 117 aa, synthetic construct
  REGION 1..117: note = SIRPa truncated mutant-m12N
ELQVIQPDKSVVVAAGETATLRCTATSLFPVGPIQWFRGAGPGRILIYNRRQGHFPRVTTVSDLTKRNNMDFSIRIGAITPADAGTYYCVKFRKGSPDDIEFKSGAGTELSVRAKPS

SEQ ID NO: 2 - protein, 117 aa, synthetic construct
  REGION 1..117: note = SIRPa truncated wildtype
ELQVIQPDKSVLVAAGETATLRCTATSLIPVGPIQWFRGAGPGRELIYNQKEGHFPRVTTVSDLTKRNNMDFSIRIGNITPADAGTYYCVKFRKGSPDDVEFKSGAGTELSVRAKPS

SEQ ID NO: 3 - protein, 504 aa, synthetic construct
  REGION 1..504: note = human SIRPa variant 1
MEPAGPAPGRLGPLLCLLLAASCAWSGVAGEEELQVIQPDKSVLVAAGETATLRCTATSLIPVGPIQWFRGAGPGRELIYNQKEGHFPRVTTVSDLTKRNNMDFSIRIGNITPADAGTYYCVKFRKGSPDDVEFKSGAGTELSVRAKPSAPVVSGPAARATPQHTVSFTCESHGFSPRDITLKWFKNGNELSDFQTNVDPVGESVSYSIHSTAKVVLTREDVHSQVICEVAHVTLQGDPLRGTANLSETIRVPPTLEVTQQPVRAENQVNVTCQVRKFYPQRLQLTWLENGNVSRTETASTVTENKDGTYNWMSWLLVNVSAHRDDVKLTCQVEHDGQPAVSKSHDLKVSAHPKEQGSNTAAENTGSNERNIYIVVGVVCTLLVALLMAALYLVRIRQKKAQGSTSSTRLHEPEKNAREITQDTNDITYADLNLPKGKKPAPQAAEPNNHTEYASIQTSPQPASEDTLTYADLDMVHLNRTPKQPAPKPEPSFSEYASVQVPRK

SEQ ID NO: 4 - protein, 232 aa, synthetic construct
  REGION 1..232: note = IgG1-Fc
EPKSCDKTHTCPPCPAPELLGGPSVFLFPPKPKDTLMISRTPEVTCVVVDVSHEDPEVKFNWYVDGVEVHNAKTKPREEQYNSTYRVVSVLTVLHQDWLNGKEYKCKVSNKALPAPIEKTISKAKGQPREPQVYTLPPSRDELTKNQVSLTCLVKGFYPSDIAVEWESNGQPENNYKTTPPVLDSDGSFFLYSKLTVDKSRWQQGNVFSCSVMHEALHNHYTQKSLSLSPGK

SEQ ID NO: 5 - protein, 229 aa, synthetic construct
  REGION 1..229: note = IgG4-Fc
ESKYGPPCPPCPAPEFLGGPSVFLFPPKPKDTLMISRTPEVTCVVVDVSQEDPEVQFNWYVDGVEVHNAKTKPREEQFNSTYRVVSVLTVLHQDWLNGKEYKCKVSNKGLPSSIEKTISKAKGQPREPQVYTLPPSQEEMTKNQVSLTCLVKGFYPSDIAVEWESNGQPENNYKTTPPVLDSDGSFFLYSRLTVDKSRWQEGNVFSCSVMHEALHNHYTQKSLSLSLGK

SEQ ID NO: 6 - protein, 349 aa, synthetic construct
  REGION 1..349: note = m12N-Fc (IgG1)
ELQVIQPDKSVVVAAGETATLRCTATSLFPVGPIQWFRGAGPGRILIYNRRQGHFPRVTTVSDLTKRNNMDFSIRIGAITPADAGTYYCVKFRKGSPDDIEFKSGAGTELSVRAKPSEPKSCDKTHTCPPCPAPELLGGPSVFLFPPKPKDTLMISRTPEVTCVVVDVSHEDPEVKFNWYVDGVEVHNAKTKPREEQYNSTYRVVSVLTVLHQDWLNGKEYKCKVSNKALPAPIEKTISKAKGQPREPQVYTLPPSRDELTKNQVSLTCLVKGFYPSDIAVEWESNGQPENNYKTTPPVLDSDGSFFLYSKLTVDKSRWQQGNVFSCSVMHEALHNHYTQKSLSLSPGK

SEQ ID NO: 7 - protein, 346 aa, synthetic construct
  REGION 1..346: note = m12N-Fc (IgG4)
ELQVIQPDKSVVVAAGETATLRCTATSLFPVGPIQWFRGAGPGRILIYNRRQGHFPRVTTVSDLTKRNNMDFSIRIGAITPADAGTYYCVKFRKGSPDDIEFKSGAGTELSVRAKPSESKYGPPCPPCPAPEFLGGPSVFLFPPKPKDTLMISRTPEVTCVVVDVSQEDPEVQFNWYVDGVEVHNAKTKPREEQFNSTYRVVSVLTVLHQDWLNGKEYKCKVSNKGLPSSIEKTISKAKGQPREPQVYTLPPSQEEMTKNQVSLTCLVKGFYPSDIAVEWESNGQPENNYKTTPPVLDSDGSFFLYSRLTVDKSRWQEGNVFSCSVMHEALHNHYTQKSLSLSLGK

SEQ ID NO: 8 - protein, 117 aa, synthetic construct
  REGION 1..117: note = m1N
ELQVIQPDKSVLVAAGETATLRCTATSLLPIGPIQWFRGAGPGRILIYNQKKGHFPRVTTLSDSTRRGNMDFSIRIGAITPADAGTYYCVKFRKGSPDDLEFKSGAGTELSVRAKPS

SEQ ID NO: 9 - protein, 117 aa, synthetic construct
  REGION 1..117: note = M5N
ELQVIQPDKSVLVAAGETATLRCTATSLVPVGPIQWFRGAGPGRNLIYNSRHGHFPRVTTVSDLTKRNNMDFSIRIGAITPADAGTYYCVKFRKGSPDDVEFKSGAGTELSVRAKPS

SEQ ID NO: 10 - protein, 117 aa, synthetic construct
  REGION 1..117: note = m170N
ELQVIQPDKSVLVAAGETATLRCTATSLFPIGPIQWFRGAGPGRELIYNQRKGHFPRVTTVSDLTKRNNMDFSIRIGAITPADAGTYYCVKFRKGSPDDIEFKSGAGTELSVRAKPS

SEQ ID NO: 11 - protein, 117 aa, synthetic construct
  REGION 1..117: note = m35N
ELQVIQPDKSVLVAAGETATLRCTATSLLPVGPIQWFRGAGPGRQLIYNQKDGHFPRVTTVSDLTKRNNMDFSINIGAITPADAGTYYCVKFRKGSPDDIEFKSGAGTELSVRAKPS

SEQ ID NO: 12 - protein, 117 aa, synthetic construct
  REGION 1..117: note = m37N
ELQVIQPDKSVLVAAGETATLRCTATSLLPIGPIQWFRGAGPGRKLIYNQRDGHFPRVTTVSDLTKRGNMDFSIRIGAITPADAGTYYCVKFRKGSPDDVEFKSGAGTELSVRAKPS

SEQ ID NO: 13 - protein, 117 aa, synthetic construct
  REGION 1..117: note = m41N
ELQVIQPDKSVLVAAGETATLRCTATSLVPVGPIQWFRGAGPGRHLIYNRRHGHFPRVTTVSDLTKRNNMDFSISIGAITPADAGTYYCVKFRKGSPDDVEFKSGAGTELSVRAKPS

SEQ ID NO: 14 - protein, 117 aa, synthetic construct
  REGION 1..117: note = m57N
ELQVIQPDKSVLVAAGETATLRCTATSLLPVGPIQWFRGAGPGRILIYNGKRGHFPRVTTLSDTTKRGNMDFSISIRAITPADAGTYYCVKFRKGSPDDREFKSGAGTELSVRAKPS

SEQ ID NO: 15 - protein, 117 aa, synthetic construct
  REGION 1..117: note = m67N
ELQVIQPDKSVLVAAGETATLRCTATSLLPVGPIQWFRGAGPGRMLIYNGRDGHFPRVTTVSDLTKRNNMDFSIRIGAITPADAGTYYCVKFRKGSPDDLEFKSGAGTELSVRAKPS

SEQ ID NO: 16 - protein, 117 aa, synthetic construct
  REGION 1..117: note = m81N
ELQVIQPDKSVLVAAGETATLRCTATSLLPVGPIQWFRGAGPGRELIYNQKEGHFPRVTTVSDLTKRNNMDFSIRIGAITPADAGTYYCVKFRKGSPDDVEFKSGAGTELSVRAKPS

SEQ ID NO: 17 - protein, 117 aa, synthetic construct
  REGION 1..117: note = m82N
ELQVIQPDKSVLVAAGETATLRCTATSLFPVGPIQWFRGAGPGRELIYNQKEGHFPRVTTVSHSTKRNNMDFSIRIHAITPADAGTYYCVKFRKGSPDDSEFKSGAGTELSVRAKPS

SEQ ID NO: 18 - protein, 117 aa, synthetic construct
  REGION 1..117: note = m84N
ELQVIQPDKSVLVAAGETATLRCTATSLFPVGPIQWFRGAGPGRELIYNQKEGHFPRVTTVSHSTRRNNMDFSIRIHAITPADAGTYYCVKFRKGSPDDSEFKSGAGTELSVRAKPS

SEQ ID NO: 19 - protein, 117 aa, synthetic construct
  REGION 1..117: note = m91N
ELQVIQPDKSVLVAAGETATLRCTATSLLPVGPIQWFRGAGPGRQLIYNQKDGHFPRVTTASDLTKRNNMDFSINIGAITPADAGTYYCVKFRKGSPDDIEFKSGAGTELSVRAKPS

SEQ ID NO: 20 - protein, 117 aa, synthetic construct
  REGION 1..117: note = m99N
ELQVIQPDKSVLVAAGETATLRCTATSLIPVGPIQWFRGAGPGRKLIYNQKEGHFPRVTTVSDSTKRKNMDFSIRIHAITPADAGTYYCVKFRKGSPDDLEFKSGAGTELSVRAKPS

SEQ ID NO: 21 - protein, 117 aa, synthetic construct
  REGION 1..117: note = m102N
ELQVIQPDKSVLVAAGETATLRCTATSLLPIGPIQWFRGAGPGRELIYNGKGGHFPRVTTVSRSTKRDNMDFSIRIGAITPADAGTYYCVKFRKGSPDDIEFKSGAGTELSVRAKPS

SEQ ID NO: 22 - protein, 117 aa, synthetic construct
  REGION 1..117: note = m111N
ELQVIQPDKSVLVAAGETATLRCTATSLLPVGPIQWFRGAGPGRRLIYNNRGGHFPRVTTLSETTRRDNMDFSIRIGAITPADAGTYYCVKFRKGSPDDLEFKSGAGTELSVRAKPS

SEQ ID NO: 23 - protein, 117 aa, synthetic construct
  REGION 1..117: note = m122N
ELQVIQPDKSVLVAAGETATLRCTATSLVPVGPIQWFRGAGPGRNLIYNSRHGHFPRVTTASDLTKRNNMDFSIRIGAITPADAGTYYCVKFRKGSPDDVEFKSGAGTELSVRAKPS

SEQ ID NO: 24 - protein, 117 aa, synthetic construct
  REGION 1..117: note = m126N
ELQVIQPDKSVLVAAGETATLRCTATSLVPIGPIQWFRGAGPGRVLIYNQRDGHFPRVTTVSETTRRENMDFSIRIGAITPADAGTYYCVKFRKGSPDDVEFKSGAGTELSVRAKPS

SEQ ID NO: 25 - protein, 117 aa, synthetic construct
  REGION 1..117: note = m130N
ELQVIQPDKSVLVAAGETATLRCTATSLLPIGPIQWFRGAGPGRVLIYNQREGHFPRVTTVSESTRRDNMDFSIRIRAITPADAGTYYCVKFRKGSPDDVEFKSGAGTELSVRAKPS

SEQ ID NO: 26 - protein, 117 aa, synthetic construct
  REGION 1..117: note = m135N
ELQVIQPDKSVLVAAGETATLRCTATSLVPVGPIQWFRGAGPGRLLIYNGKGGHFPRVTTLSETTRRGNMDFSIRIGAITPADAGTYYCVKFRKGSPDDVEFKSGAGTELSVRAKPS

SEQ ID NO: 27 - protein, 117 aa, synthetic construct
  REGION 1..117: note = m145N
ELQVIQPDKSVLVAAGETATLRCTATSLLPIGPIQWFRGAGPGRNLIYNGKGGHFPRVTTVSDLTKRNNMDFSIRIGAITPADAGTYYCVKFRKGSPDDVEFKSGAGTELSVRAKPS